European Patent Specification EP 3 658 668 B1, published December 11, 2024. Title: Adenoviral Vectors. Applicant: Oxford Genetics Limited. The sequence listing filed with the application follows.

SEQUENCE LISTING (18 sequences)

SEQ ID NO: 1 - DNA, 107 bp, Human adenovirus type 5
cgccctcttcggcatcaaggaaggtgattggtttgtaggtgtaggccacgtgaccgggtgttcctgaaggggggctataaaagggggtgggggcgcgttcgtcctca

SEQ ID NO: 2 - DNA, 19 bp, Artificial Sequence
  TetR binding site
tccctatcagtgatagaga

SEQ ID NO: 3 - DNA, 624 bp, Artificial Sequence
  TetR
atgtcgcgcctggacaaaagcaaagtgattaactcagcgctggaactgttgaatgaggtgggaattgaaggactcactactcgcaagctggcacagaagctgggcgtcgagcagccaacgctgtactggcatgtgaagaataaacgggcgctcctagacgcgcttgccatcgaaatgctggaccgccatcacacccacttttgccccctggagggcgaatcctggcaagattttctgcggaacaatgcaaagtcgttccggtgcgctctgctgtcccaccgcgatggcgcaaaagtgcacctgggcactcggcccaccgagaaacaatacgaaaccctggaaaaccaactggctttcctttgccaacagggattttcactggagaatgccctgtacgcactatccgcggtcggccactttaccctgggatgcgtcctcgaagatcaggagcaccaagtcgccaaggaggaaagagaaactcctaccactgactcaatgcctccgctcctgagacaagccatcgagctgttcgaccaccagggtgctgaacctgcatttctgttcgggcttgaactgattatctgcggcctggagaaacagttgaagtgcgagtcgggatcctag

SEQ ID NO: 4 - protein, 207 aa, Artificial Sequence
  TetR
MSRLDKSKVINSALELLNEVGIEGLTTRKLAQKLGVEQPTLYWHVKNKRALLDALAIEMLDRHHTHFCPLEGESWQDFLRNNAKSFRCALLSHRDGAKVHLGTRPTEKQYETLENQLAFLCQQGFSLENALYALSAVGHFTLGCVLEDQEHQVAKEERETPTTDSMPPLLRQAIELFDHQGAEPAFLFGLELIICGLEKQLKCESGS

SEQ ID NO: 5 - protein, 8 aa, Artificial Sequence
  Opposite TetR binding site
ESLSLIGT

SEQ ID NO: 6 - DNA, 107 bp, Artificial Sequence
  Modified MLP
cgccctcttcggcatcaaggaaggtgattggtttgtaggtgtaggccacgtgaccgggtgttcctgaaggggggctataaaaggtccctatcagtgatagagactca

SEQ ID NO: 7 - DNA, 107 bp, Artificial Sequence
  Modified MLP
cgccctcttcggcatcaaggaaggtgattggtttgtaggtgtaggccacgtgactccctatcagtgatagagaactataaaaggtccctatcagtgatagagactca

SEQ ID NO: 8 - DNA, 416 bp, Artificial Sequence
  Sequence in viral vector or other sequence
aggccagcacgaaggaggctaagtgggaggggtagcggtcgttgtccactagggggtccactcgctccagggtgtgaagacacatgtcgccctcttcggcatcaaggaaggtgattggtttgtaggtgtaggccacgtgaccgggtgttcctgaaggggggctataaaaggtccctatcagtgatagagactcactctcttccgcatcgctgtctgcgagggccagctgttggggtgagtactccctctgaaaagcgggcatgacttctgcgctaagattgtcagtttccaaaaacgaggaggatttgatattcacctggcccgcggtgatgcctttgagggtggccgcatccatctggtcagaaaagacaatctttttgttgtcaagcttggtggcaaacgacccgtagagggcg

SEQ ID NO: 9 - DNA, 21 bp, Artificial Sequence
  Ad5 fiber forward primer
tggctgttaaaggcagtttgg

SEQ ID NO: 10 - DNA, 23 bp, Artificial Sequence
  Ad5 fiber reverse primer
gcactccattttcgtcaaatctt

SEQ ID NO: 11 - DNA, 33 bp, Artificial Sequence
  TaqMan probe
tccaatatctggaacagttcaaagtgctcatct

SEQ ID NO: 12 - protein, 173 aa, Human adenovirus type 5
IAKLLSNALYGSFATKLDNKKIVFSDQMDAATLKGITAGQVNIKSSSFLETDNLSAEVMPAFQREYSPQQLALADSDAEESEDERAPTPFYSPPSGTPGHVAYTYKPITFLDAEEGDMCLHTLERVDPLVDNDRYPSHLASFVLAWTRAFVSEWSEFLYEEDRGTPLEDRPLK

SEQ ID NO: 13 - DNA, 390 bp, Human adenovirus type 5
cactagggggtccactcgctccagggtgtgaagacacatgtcgccctcttcggcatcaaggaaggtgattggtttgtaggtgtaggccacgtgaccgggtgttcctgaaggggggctataaaagggggtgggggcgcgttcgtcctcactctcttccgcatcgctgtctgcgagggccagctgttggggtgagtactccctctgaaaagcgggcatgacttctgcgctaagattgtcagtttccaaaaacgaggaggatttgatattcacctggcccgcggtgatgcctttgagggtggccgcatccatctggtcagaaaagacaatctttttgttgtcaagcttggtggcaaacgacccgtagagggcgttggacagcaacttggcgat

SEQ ID NO: 14 - DNA, 390 bp, Human adenovirus type 5
atcgccaagttgctgtccaacgccctctacgggtcgtttgccaccaagcttgacaacaaaaagattgtcttttctgaccagatggatgcggccaccctcaaaggcatcaccgcgggccaggtgaatatcaaatcctcctcgtttttggaaactgacaatcttagcgcagaagtcatgcccgcttttcagagggagtactcaccccaacagctggccctcgcagacagcgatgcggaagagagtgaggacgaacgcgcccccacccccttttatagccccccttcaggaacacccggtcacgtggcctacacctacaaaccaatcaccttccttgatgccgaagagggcgacatgtgtcttcacaccctggagcgagtggaccccctagtg

SEQ ID NO: 15 - protein, 160 aa, Artificial Sequence
  Modified MLP
AKERADRDKNQTLRSIAKLLSNALYGSFATKLDNKKIVFSDQMDAATLKGITAGQVNIKSSSFLETDNLSAEVMPAFQREYSPQQLALADSDAEESESLSLIGTFYSPPSGTPGHVAYTYKPITFLDAEEGDMCLHTLERVDPLVDNDRYPSHLASFVLA

SEQ ID NO: 16 - DNA, 480 bp, Artificial Sequence
  Modified MLP
aggccagcacgaaggaggctaagtgggaggggtagcggtcgttgtccactagggggtccactcgctccagggtgtgaagacacatgtcgccctcttcggcatcaaggaaggtgattggtttgtaggtgtaggccacgtgaccgggtgttcctgaaggggggctataaaaggtccctatcagtgatagagactcactctcttccgcatcgctgtctgcgagggccagctgttggggtgagtactccctctgaaaagcgggcatgacttctgcgctaagattgtcagtttccaaaaacgaggaggatttgatattcacctggcccgcggtgatgcctttgagggtggccgcatccatctggtcagaaaagacaatctttttgttgtcaagcttggtggcaaacgacccgtagagggcgttggacagcaacttggcgatggagcgcagggtttggtttttgtcgcgatcggcgcgctccttgg

SEQ ID NO: 17 - DNA, 480 bp, Artificial Sequence
  Modified MLP
ccaaggagcgcgccgatcgcgacaaaaaccaaaccctgcgctccatcgccaagttgctgtccaacgccctctacgggtcgtttgccaccaagcttgacaacaaaaagattgtcttttctgaccagatggatgcggccaccctcaaaggcatcaccgcgggccaggtgaatatcaaatcctcctcgtttttggaaactgacaatcttagcgcagaagtcatgcccgcttttcagagggagtactcaccccaacagctggccctcgcagacagcgatgcggaagagagtgagtctctatcactgatagggaccttttatagccccccttcaggaacacccggtcacgtggcctacacctacaaaccaatcaccttccttgatgccgaagagggcgacatgtgtcttcacaccctggagcgagtggaccccctagtggacaacgaccgctacccctcccacttagcctccttcgtgctggcct

SEQ ID NO: 18 - protein, 8 aa, Artificial Sequence
  DNA polymerase coding sequence between MLP TATA box and +1
ENERAPTP